European Patent Application EP 4 759 807 A1, published June 17, 2026. Title: 一种降解 IRAK4 的蛋白降解靶向嵌合体化合物及其应用. Applicant: 深圳众格生物科技有限公司. The sequence listing filed with the application follows.

SEQUENCE LISTING (2 sequences)

SEQ ID NO: 1 - DNA, 33 bp, synthetic construct
  source 1..33: mol_type = other DNA
gtgagcggctggcggctgttcaagaagattagc

SEQ ID NO: 2 - DNA, 1422 bp, synthetic construct
  source 1..1422: mol_type = other DNA
gccaccatgaacaaacccataacaccatcaacatatgtgcgctgcctcaatgttggactaattaggaagctgtcagattttattgatcctcaagaaggatggaagaagttagctgtagctattaaaaaaccatctggtgatgatagatacaatcagtttcacataaggagatttgaagcattacttcaaactggaaaaagtcccacttctgaattactgtttgactggggcaccacaaattgcacagttggtgatcttgtggatcttttgatccaaaatgaattttttgctcctgcgagtcttttgctcccagatgctgttcccaaaactgctaatacactaccttctaaagaagctataacagttcagcaaaaacagatgcctttctgtgacaaagacaggacattgatgacacctgtgcagaatcttgaacaaagctatatgccacctgactcctcaagtccagaaaataaaagtttagaagttagtgatacacgttttcacagtttttcattttatgaattgaagaatgtcacaaataactttgatgaacgacccatttctgttggtggtaataaaatgggagagggaggatttggagttgtatataaaggctacgtaaataacacaactgtggcagtgaagaagcttgcagcaatggttgacattactactgaagaactgaaacagcagtttgatcaagaaataaaagtaatggcaaagtgtcaacatgaaaacttagtagaactacttggtttctcaagtgatggagatgacctctgcttagtatatgtttacatgcctaatggttcattgctagacagactctcttgcttggatggtactccaccactttcttggcacatgagatgcaagattgctcagggtgcagctaatggcatcaattttctacatgaaaatcatcatattcatagagatattaaaagtgcaaatatcttactggatgaagcttttactgctaaaatatctgactttggccttgcacgggcttctgagaagtttgcccagacagtcatgactagcagaattgtgggaacaacagcttatatggcaccagaagctttgcgtggagaaataacacccaaatctgatatttacagctttggtgtggttttactagaaataataactggacttccagctgtggatgaacaccgtgaacctcagttattgctagatattaaagaagaaattgaagatgaagaaaagacaattgaagattatattgataaaaagatgaatgatgctgattccacttcagttgaagctatgtactctgttgctagtcaatgtctgcatgaaaagaaaaataagagaccagacattaagaaggttcaacagctgctgcaagagatgacagcttctgtgagcggctggcggctgttcaagaagattagctaa